European Patent Application EP 4 219 541 A2, published August 2, 2023. Title: T Cell Receptors. Applicant: Immunocore Limited. The sequence listing filed with the application follows.

SEQUENCE LISTING (64 sequences)

SEQ ID NO: 1 - protein, 9 aa, Homo sapiens
SLLQHLIGL

SEQ ID NO: 2 - protein, 200 aa, Homo sapiens
DAKTTQPNSMESNEEEPVHLPCNHSTISGTDYIHWYRQLPSQGPEYVIHGLTSNVNNRMASLAIAEDRKSSTLILHRATLRDAAVYYCILILGHSGAGSYQLTFGKGTKLSVIPNIQNPDPAVYQLRDSKSSDKSVCLFTDFDSQTNVSQSKDSDVYITDKTVLDMRSMDFKSNSAVAWSNKSDFACANAFNNSIIPEDT

SEQ ID NO: 3 - protein, 244 aa, Homo sapiens
DGGITQSPKYLFRKEGQNVTLSCEQNLNHDAMYWYRQDPGQGLRLIYYSQIVNDFQKGDIAEGYSVSREKKESFPLTVTSAQKNPTAFYLCASSPWTSGSREQYFGPGTRLTVTEDLKNVFPPEVAVFEPSEAEISHTQKATLVCLATGFYPDHVELSWWVNGKEVHSGVSTDPQPLKEQPALNDSRYCLSSRLRVSATFWQNPRNHFRCQVQFYGLSENDEWTQDRAKPVTQIVSAEAWGRAD

SEQ ID NO: 4 - protein, 200 aa, Homo sapiens
DAKTTQPNSMESNEEEPVHLPCNHSTISGTDYIHWYRQLPSQGPEYVIHGLTSNVNNRMASLAIAEDRKSSTLILHRATLRDAAVYYCILILGHSGAGSYQLTFGKGTKLSVIPNIQNPDPAVYQLRDSKSSDKSVCLFTDFDSQTNVSQSKDSDVYITDKCVLDMRSMDFKSNSAVAWSNKSDFACANAFNNSIIPEDT

SEQ ID NO: 5 - protein, 244 aa, Homo sapiens
DGGITQSPKYLFRKEGQNVTLSCEQNLNHDAMYWYRQDPGQGLRLIYYSQIVNDFQKGDIAEGYSVSREKKESFPLTVTSAQKNPTAFYLCASSPWTSGSREQYFGPGTRLTVTEDLKNVFPPEVAVFEPSEAEISHTQKATLVCLATGFYPDHVELSWWVNGKEVHSGVCTDPQPLKEQPALNDSRYALSSRLRVSATFWQDPRNHFRCQVQFYGLSENDEWTQDRAKPVTQIVSAEAWGRAD

SEQ ID NO: 6 - protein, 115 aa, Homo sapiens
GDAKTTQPNSMESNEEEPVHLPCNHSTISGTDYIHWYRQLPSQGPEYVIHGLTSNVNNRMASLAIAEDRKSSTLILHRATLRDAAVYYCILILGHSRAGNYIATFGKGTKLSVIP

SEQ ID NO: 7 - protein, 115 aa, Homo sapiens
GDAKTTQPNSMESNEEEPVHLPCNHSTISGTDYIHWYRQLPSQGPEYVIHGLTSNVNNRMASLAIAEDRKSSTLILHRATLRDAAVYYCILILGHSRLGNYIATFGKGTKLSVIP

SEQ ID NO: 8 - protein, 115 aa, Homo sapiens
GDAKTTQPNSMESNEEEPVHLPCNHSTISGTDYIHWYRQLPSQGPEYVIHGLTSNVNNRMASLAIAEDRKSSTLILHRATLRDAAVYYCILILGHSRLGNYQATFGKGTKLSVIP

SEQ ID NO: 9 - protein, 114 aa, Homo sapiens
DGGITQSPKYLFRKEGQNVTLSCEQNLNHDAMYWYRQDPGQGLRLIYYSQIMGDEQKGDIAEGYSVSREKKESFPLTVTSAQKNPTAFYLCASSWWTGGASPISFGPGTRLTVT

SEQ ID NO: 10 - protein, 114 aa, Homo sapiens
DGGITQSPKYLFRKEGQNVTLSCEQNLNHDAMYWYRQDPGQGLRLIYYSQIMGDEQKGDIAEGYSVSREKKESFPLTVTSAQKNPTAFYLCASSWWTSGASPISFGPGTRLTVT

SEQ ID NO: 11 - protein, 114 aa, Homo sapiens
DGGITQSPKYLFRKEGQNVTLSCEQNLNHDAMYWYRQDPGQGLRLIYYSQIMGDEQKGDIAEGYSVSREKKESFPLTVTSAQKNPTAFYLCASSWWTGGSAPIRFGPGTRLTVT

SEQ ID NO: 12 - protein, 114 aa, Homo sapiens
DGGITQSPKYLFRKEGQNVTLSCEQNLNHDAMYWYRQDPGQGLRLIYYSQIMNDEQKGDIAEGYSVSREKKESFPLTVTSAQKNPTAFYLCASSWWTGGSAPIRFGPGTRLTVT

SEQ ID NO: 13 - protein, 114 aa, Homo sapiens
DGGITQSPKYLFRKEGQNVTLSCEQNLNHDAMYWYRQDPGQGLRLIYYSQIMGDEQKGDIAEGYSVSREKKESFPLTVTSAQKNPTAFYLCASSWWTSGSAPIRFGPGTRLTVT

SEQ ID NO: 14 - protein, 114 aa, Homo sapiens
DGGITQSPKYLFRKEGQNVTLSCEQNLNHDAMYWYRQDPGQGLRLIYYSQIMGDEQKGDIAEGYSVSREKKESFPLTVTSAQKNPTAFYLCASSWWTGGSAEIRFGPGTRLTVT

SEQ ID NO: 15 - protein, 114 aa, Homo sapiens
DGGITQSPKYLFRKEGQNVTLSCEQNLNHDAMYWYRQDPGQGLRLIYYSQIMGDEQKGDIAEGYSVSREKKESFPLTVTSAQKNPTAFYLCASSWWTGGSAPIYFGPGTRLTVT

SEQ ID NO: 16 - protein, 114 aa, Homo sapiens
DGGITQSPKYLFRKEGQNVTLSCEQNLNHDAMYWYRQDPGQGLRLIYYSQIMGDEQKGDIAEGYSVSREKKESFPLTVTSAQKNPTAFYLCASSWWTGGAAPISFGPGTRLTVT

SEQ ID NO: 17 - protein, 114 aa, Homo sapiens
DGGITQSPKYLFRKEGQNVTLSCEQNLNHDAMYWYRQDPGQGLRLIYYSQIMGDEQKGDIAEGYSVSREKKESFPLTVTSAQKNPTAFYLCASSWWTGGASPIRFGPGTRLTVT

SEQ ID NO: 18 - protein, 114 aa, Homo sapiens
DGGITQSPKYLFRKEGQNVTLSCEQNLNHDAMYWYRQDPGQGLRLIYYSQIMGDEQKGDIAEGYSVSREKKESFPLTVTSAQKNPTAFYLCASSWWTGGAAPIRFGPGTRLTVT

SEQ ID NO: 19 - protein, 114 aa, Homo sapiens
DGGITQSPKYLFRKEGQNVTLSCEQNLNHDAMYWYRQDPGQGLRLIYYSQIMGDEQKGDIAEGYSVSREKKESFPLTVTSAQKNPTAFYLCASSWWTGGASEISFGPGTRLTVT

SEQ ID NO: 20 - protein, 114 aa, Homo sapiens
DGGITQSPKYLFRKEGQNVTLSCEQNLNHDAMYWYRQDPGQGLRLIYYSQIMGDEQKGDIAEGYSVSREKKESFPLTVTSAQKNPTAFYLCASSWWTGGSAPISFGPGTRLTVT

SEQ ID NO: 21 - protein, 114 aa, Homo sapiens
DGGITQSPKYLFRKEGQNVTLSCEQNLNHDAMYWYRQDPGQGLRLIYYSQIMGDEQKGDIAEGYSVSREKKESFPLTVTSAQKNPTAFYLCASSWWTGGSSPISFGPGTRLTVT

SEQ ID NO: 22 - protein, 114 aa, Homo sapiens
DGGITQSPKYLFRKEGQNVTLSCEQNLNHDAMYWYRQDPGQGLRLIYYSQIVGDEQKGDIAEGYSVSREKKESFPLTVTSAQKNPTAFYLCASSWWTGGSAPIRFGPGTRLTVT

SEQ ID NO: 23 - protein, 114 aa, Homo sapiens
DGGITQSPKYLFRKEGQNVTLSCEQNLNHDAMYWYRQDPGQGLRLIYYSQIMGDEQKGDIAEGYSVSREKKESFPLTVTSAQKNPTAFYLCASSPWTGGSAPIRFGPGTRLTVT

SEQ ID NO: 24 - protein, 114 aa, Homo sapiens
DGGITQSPKYLFRKEGQNVTLSCEQNLNHDAMYWYRQDPGQGLRLIYYSQIMGDEQKGDIAEGYSVSREKKESFPLTVTSAQKNPTAFYLCASSWWTGGSSPIRFGPGTRLTVT

SEQ ID NO: 25 - protein, 201 aa, Homo sapiens
GDAKTTQPNSMESNEEEPVHLPCNHSTISGTDYIHWYRQLPSQGPEYVIHGLTSNVNNRMASLAIAEDRKSSTLILHRATLRDAAVYYCILILGHSRAGNYIATFGKGTKLSVIPNIQNPDPAVYQLRDSKSSDKSVCLFTDFDSQTNVSQSKDSDVYITDKCVLDMRSMDFKSNSAVAWSNKSDFACANAFNNSIIPEDT

SEQ ID NO: 26 - protein, 502 aa, Homo sapiens
AIQMTQSPSSLSASVGDRVTITCRASQDIRNYLNWYQQKPGKAPKLLIYYTSRLESGVPSRFSGSGSGTDYTLTISSLQPEDFATYYCQQGNTLPWTFGQGTKVEIKGGGGSGGGGSGGGGSGGGGSGGGSEVQLVESGGGLVQPGGSLRLSCAASGYSFTGYTMNWVRQAPGKGLEWVALINPYKGVSTYNQKFKDRFTISVDKSKNTAYLQMNSLRAEDTAVYYCARSGYYGDSDWYFDVWGQGTLVTVSSGGGGSDGGITQSPKYLFRKEGQNVTLSCEQNLNHDAMYWYRQDPGQGLRLIYYSQIMGDEQKGDIAEGYSVSREKKESFPLTVTSAQKNPTAFYLCASSWWTGGASPISFGPGTRLTVTEDLKNVFPPEVAVFEPSEAEISHTQKATLVCLATGFYPDHVELSWWVNGKEVHSGVCTDPQPLKEQPALNDSRYALSSRLRVSATFWQDPRNHFRCQVQFYGLSENDEWTQDRAKPVTQIVSAEAWGRAD

SEQ ID NO: 27 - protein, 201 aa, Homo sapiens
GDAKTTQPNSMESNEEEPVHLPCNHSTISGTDYIHWYRQLPSQGPEYVIHGLTSNVNNRMASLAIAEDRKSSTLILHRATLRDAAVYYCILILGHSRLGNYIATFGKGTKLSVIPNIQNPDPAVYQLRDSKSSDKSVCLFTDFDSQTNVSQSKDSDVYITDKCVLDMRSMDFKSNSAVAWSNKSDFACANAFNNSIIPEDT

SEQ ID NO: 28 - protein, 502 aa, Homo sapiens
AIQMTQSPSSLSASVGDRVTITCRASQDIRNYLNWYQQKPGKAPKLLIYYTSRLESGVPSRFSGSGSGTDYTLTISSLQPEDFATYYCQQGNTLPWTFGQGTKVEIKGGGGSGGGGSGGGGSGGGGSGGGSEVQLVESGGGLVQPGGSLRLSCAASGYSFTGYTMNWVRQAPGKGLEWVALINPYKGVSTYNQKFKDRFTISVDKSKNTAYLQMNSLRAEDTAVYYCARSGYYGDSDWYFDVWGQGTLVTVSSGGGGSDGGITQSPKYLFRKEGQNVTLSCEQNLNHDAMYWYRQDPGQGLRLIYYSQIMGDEQKGDIAEGYSVSREKKESFPLTVTSAQKNPTAFYLCASSWWTGGASPIRFGPGTRLTVTEDLKNVFPPEVAVFEPSEAEISHTQKATLVCLATGFYPDHVELSWWVNGKEVHSGVCTDPQPLKEQPALNDSRYALSSRLRVSATFWQDPRNHFRCQVQFYGLSENDEWTQDRAKPVTQIVSAEAWGRAD

SEQ ID NO: 29 - protein, 201 aa, Homo sapiens; identical to SEQ ID NO: 27

SEQ ID NO: 30 - protein, 501 aa, Homo sapiens
AIQMTQSPSSLSASVGDRVTITCRASQDIRNYLNWYQQKPGKAPKLLIYYTSRLESGVPSRFSGSGSGTDYTLTISSLQPEDFATYYCQQGNTLPWTFGQGTKVEIKGGGGSGGGGSGGGGSGGGGSGGGSEVQLVESGGGLVQPGGSLRLSCAASGYSFTGYTMNWVRQAPGKGLEWVALINPYKGVSTYNQKFKDRFTISVDKSKNTAYLQMNSLRAEDTAVYYCARSGYYGDSDWYFDVWGQGTLVTVSSGGGGSDGGITQSPKYLFRKEGQNVTLSCEQNLNHDAMYWYRQDPGQGLRLIYYSQIMGDEQKGDIAEGYSVSREKKESFPLTVTSAQKNPTAFYLCASSWWTGGSAPIRFGPGTRLTVTEDLKNVFPPEVAVFEPSEAEISHTQKATLVCLATGFYPDHVELSWWVNGKEVHSGVCTDPQPLKEQPALNDSRYALSSRLRVSATFWQDPRNHFRCQVQFYGLSENDEWTQDRAKPVTQIVSAEAWGRA

SEQ ID NO: 31 - protein, 5 aa, Homo sapiens
GGGGS

SEQ ID NO: 32 - protein, 5 aa, Homo sapiens
GGGSG

SEQ ID NO: 33 - protein, 5 aa, Homo sapiens
GGSGG

SEQ ID NO: 34 - protein, 5 aa, Homo sapiens
GSGGG

SEQ ID NO: 35 - protein, 6 aa, Homo sapiens
GSGGGP

SEQ ID NO: 36 - protein, 5 aa, Homo sapiens
GGEPS

SEQ ID NO: 37 - protein, 7 aa, Homo sapiens
GGEGGGP

SEQ ID NO: 38 - protein, 12 aa, Homo sapiens
GGEGGGSEGGGS

SEQ ID NO: 39 - protein, 7 aa, Homo sapiens
TISGTDY

SEQ ID NO: 40 - protein, 5 aa, Homo sapiens
GLTSN

SEQ ID NO: 41 - protein, 17 aa, Homo sapiens
CILILGHSGAGSYQLTF

SEQ ID NO: 42 - protein, 5 aa, Homo sapiens
LNHDA

SEQ ID NO: 43 - protein, 7 aa, Homo sapiens
SQIVNDF

SEQ ID NO: 44 - protein, 15 aa, Homo sapiens
CASSPWTSGSREQYF

SEQ ID NO: 45 - protein, 17 aa, Homo sapiens
CILILGHSRAGNYIATF

SEQ ID NO: 46 - protein, 17 aa, Homo sapiens
CILILGHSRLGNYIATF

SEQ ID NO: 47 - protein, 17 aa, Homo sapiens
CILILGHSRLGNYQATF

SEQ ID NO: 48 - protein, 7 aa, Homo sapiens
SQIMGDE

SEQ ID NO: 49 - protein, 7 aa, Homo sapiens
SQIMNDE

SEQ ID NO: 50 - protein, 7 aa, Homo sapiens
SQIVGDE

SEQ ID NO: 51 - protein, 15 aa, Homo sapiens
CASSWWTGGASPISF

SEQ ID NO: 52 - protein, 15 aa, Homo sapiens
CASSWWTSGASPISF

SEQ ID NO: 53 - protein, 15 aa, Homo sapiens
CASSWWTGGSAPIRF

SEQ ID NO: 54 - protein, 15 aa, Homo sapiens
CASSWWTSGSAPIRF

SEQ ID NO: 55 - protein, 15 aa, Homo sapiens
CASSWWTGGSAEIRF

SEQ ID NO: 56 - protein, 15 aa, Homo sapiens
CASSWWTGGSAPIYF

SEQ ID NO: 57 - protein, 15 aa, Homo sapiens
CASSWWTGGAAPISF

SEQ ID NO: 58 - protein, 15 aa, Homo sapiens
CASSWWTGGASPIRF

SEQ ID NO: 59 - protein, 15 aa, Homo sapiens
CASSWWTGGAAPIRF

SEQ ID NO: 60 - protein, 15 aa, Homo sapiens
CASSWWTGGASEISF

SEQ ID NO: 61 - protein, 15 aa, Homo sapiens
CASSWWTGGSAPISF

SEQ ID NO: 62 - protein, 15 aa, Homo sapiens
CASSWWTGGSSPISF

SEQ ID NO: 63 - protein, 15 aa, Homo sapiens
CASSPWTGGSAPIRF

SEQ ID NO: 64 - protein, 15 aa, Homo sapiens
CASSWWTGGSSPIRF